European Patent Application EP 4 790 146 A1, published August 12, 2026. Title: 可用于肿瘤鉴定的新型DNA甲基化标志物TAGMe-3及其用途. Applicant: 上海奕谱生物科技有限公司. The sequence listing filed with the application follows.

SEQUENCE LISTING (30 sequences)

SEQ ID NO: 1 - DNA, 797 bp, Homo sapiens
  source 1..797: mol_type = genomic DNA
aggtatgggtttggtgtcccgtacagcgatcgctttgtgggtttagtacttggtgctgacaaataatggagtgagatccgaacataaaggcaggcagagatgttttggggctgaatcaccgaatactagagtaggtttggggctacgtaaagacttgcttgaaaacaactaccatttagttgcgaatccctcccctcttccctttgattcgatgtttaaaaagaatcccaaatcacagttggacatactcctgccacagccttgggcagaagtcttcaaagcatgaaaagatgtggtttggcgactttgagttgtcgggtatttttgtgtcccaggagtgtgagaaaggggctacgttccgcgtcttccggaggcgcacagcaagggagtctcctggtgtcatctcgggccattacggcgcttagtcgatcattaggtctgtgggtgactgtaggcagagccgggagttgggtgcttggcgcggagggtgaactcgcgggtcttgagctgcaactagaagctgctcctagcaaggggtcgggtggagatgaaaagactgtggggaaggggaggtggttgtatgcccagagatatcccggcgtaactacggagtccaggcccagagtggcggtgtgtggcgaaggcgcagcaggcctgcgcctgtcggaggacggcagatctggacgcgaccgcgcgggcgtgcctgggtcccgcttcctgcccatcgagggcgacttccttcgggctcagctgtgagctccaggaactctgcaacctcccgacgggcgccacgctcc

SEQ ID NO: 2 - DNA, 797 bp, synthetic construct
  source 1..797: mol_type = other DNA
aggtatgggtttggtgtttygtatagygatygttttgtgggtttagtatttggtgttgataaataatggagtgagattygaatataaaggtaggtagagatgttttggggttgaattatygaatattagagtaggtttggggttaygtaaagatttgtttgaaaataattattatttagttgygaatttttttttttttttttttgattygatgtttaaaaagaattttaaattatagttggatatatttttgttatagttttgggtagaagtttttaaagtatgaaaagatgtggtttggygattttgagttgtygggtatttttgtgttttaggagtgtgagaaaggggttaygtttygygtttttyggaggygtatagtaagggagttttttggtgttatttygggttattayggygtttagtygattattaggtttgtgggtgattgtaggtagagtygggagttgggtgtttggygyggagggtgaattygygggttttgagttgtaattagaagttgtttttagtaaggggtygggtggagatgaaaagattgtggggaaggggaggtggttgtatgtttagagatatttyggygtaattayggagtttaggtttagagtggyggtgtgtggygaaggygtagtaggtttgygtttgtyggaggayggtagatttggaygygatygygygggygtgtttgggtttygttttttgtttatygagggygatttttttygggtttagttgtgagttttaggaattttgtaatttttygaygggygttaygtttt

SEQ ID NO: 3 - DNA, 58 bp, synthetic construct
  source 1..58: mol_type = other DNA
tacacgacgctcttccgatctcgtgatygtttttaaagtatgaaaagatgtggtttgg

SEQ ID NO: 4 - DNA, 57 bp, synthetic construct
  source 1..57: mol_type = other DNA
gacgtgtgctcttccgatcttagcttrctacctacaatcacccacaaacctaataat

SEQ ID NO: 5 - DNA, 58 bp, synthetic construct
  source 1..58: mol_type = other DNA
aatgatacggcgaccaccgagatctacactctttccctacacgacgctcttccgatct

SEQ ID NO: 6 - DNA, 64 bp, synthetic construct
  source 1..64: mol_type = other DNA
caagcagaagacggcatacgagatcgtgatgtgactggagttcagacgtgtgctcttccgatct

SEQ ID NO: 7 - DNA, 28 bp, synthetic construct
  source 1..28: mol_type = other DNA
tacacgacgctcttccgatctcgtgaty

SEQ ID NO: 8 - DNA, 28 bp, synthetic construct
  source 1..28: mol_type = other DNA
tacacgacgctcttccgatctacatcgy

SEQ ID NO: 9 - DNA, 28 bp, synthetic construct
  source 1..28: mol_type = other DNA
tacacgacgctcttccgatctgcctaay

SEQ ID NO: 10 - DNA, 28 bp, synthetic construct
  source 1..28: mol_type = other DNA
tacacgacgctcttccgatcttggtcay

SEQ ID NO: 11 - DNA, 28 bp, synthetic construct
  source 1..28: mol_type = other DNA
tacacgacgctcttccgatctcactgty

SEQ ID NO: 12 - DNA, 28 bp, synthetic construct
  source 1..28: mol_type = other DNA
tacacgacgctcttccgatctattggcy

SEQ ID NO: 13 - DNA, 28 bp, synthetic construct
  source 1..28: mol_type = other DNA
tacacgacgctcttccgatctgatctgy

SEQ ID NO: 14 - DNA, 28 bp, synthetic construct
  source 1..28: mol_type = other DNA
tacacgacgctcttccgatcttcaagty

SEQ ID NO: 15 - DNA, 28 bp, synthetic construct
  source 1..28: mol_type = other DNA
tacacgacgctcttccgatctctgatcy

SEQ ID NO: 16 - DNA, 28 bp, synthetic construct
  source 1..28: mol_type = other DNA
tacacgacgctcttccgatctaagctay

SEQ ID NO: 17 - DNA, 27 bp, synthetic construct
  source 1..27: mol_type = other DNA
gacgtgtgctcttccgatcttagcttr

SEQ ID NO: 18 - DNA, 27 bp, synthetic construct
  source 1..27: mol_type = other DNA
gacgtgtgctcttccgatctggctacr

SEQ ID NO: 19 - DNA, 27 bp, synthetic construct
  source 1..27: mol_type = other DNA
gacgtgtgctcttccgatctcttgtar

SEQ ID NO: 20 - DNA, 27 bp, synthetic construct
  source 1..27: mol_type = other DNA
gacgtgtgctcttccgatctagtcaar

SEQ ID NO: 21 - DNA, 27 bp, synthetic construct
  source 1..27: mol_type = other DNA
gacgtgtgctcttccgatctagttccr

SEQ ID NO: 22 - DNA, 27 bp, synthetic construct
  source 1..27: mol_type = other DNA
gacgtgtgctcttccgatctccgaccr

SEQ ID NO: 23 - DNA, 27 bp, synthetic construct
  source 1..27: mol_type = other DNA
gacgtgtgctcttccgatctggacggr

SEQ ID NO: 24 - DNA, 27 bp, synthetic construct
  source 1..27: mol_type = other DNA
gacgtgtgctcttccgatctctctacr

SEQ ID NO: 25 - DNA, 27 bp, synthetic construct
  source 1..27: mol_type = other DNA
gacgtgtgctcttccgatctgcggacr

SEQ ID NO: 26 - DNA, 27 bp, synthetic construct
  source 1..27: mol_type = other DNA
gacgtgtgctcttccgatcttgtgatr

SEQ ID NO: 27 - DNA, 25 bp, synthetic construct
  source 1..25: mol_type = other DNA
ggtatgggtttggtgtttygtatag

SEQ ID NO: 28 - DNA, 25 bp, synthetic construct
  source 1..25: mol_type = other DNA
atatccaactataatttaaaattct

SEQ ID NO: 29 - DNA, 25 bp, synthetic construct
  source 1..25: mol_type = other DNA
taggtttgtgggtgattgtaggtag

SEQ ID NO: 30 - DNA, 26 bp, synthetic construct
  source 1..26: mol_type = other DNA
aacrtaacrcccrtcraaaaattaca